European Patent Application EP 4 148 142 A1, published March 15, 2023. Title: METHODS OF SAMPLE PREPARATION. Applicant: THE SCRIPPS RESEARCH INSTITUTE. Application EP. The sequence listing filed with the application follows.

SEQUENCE LISTING (14 sequences)

SEQ ID NO: 1 - DNA, 58 bp, synthetic construct
  modified_base 58: mod_base = OTHER; note = a, c, t, g, unknown or other
  source 1..58: mol_type = other DNA
gatcggaagagcacacgtctgaactccagtcacatctcgtatgccgtcttctgcttgn

SEQ ID NO: 2 - DNA, 58 bp, synthetic construct
  modified_base 58: mod_base = OTHER; note = a, c, t, g, unknown or other
  source 1..58: mol_type = other DNA
caagcagaagacggcatacgagatgtgactggagttcagacgtgtgctcttccgatcn

SEQ ID NO: 3 - DNA, 21 bp, synthetic construct
  modified_base 14..21: mod_base = OTHER; note = a, c, t, g, unknown or other
  source 1..21: mol_type = other DNA
atcgtcgactgacnnnnnnnn

SEQ ID NO: 4 - DNA, 21 bp, synthetic construct
  modified_base 1..8: mod_base = OTHER; note = a, c, t, g, unknown or other
  source 1..21: mol_type = other DNA
nnnnnnnnctgacatcgtcga

SEQ ID NO: 5 - DNA, 95 bp, synthetic construct
  modified_base 14..21: mod_base = OTHER; note = a, c, t, g, unknown or other
  modified_base 75..82: mod_base = OTHER; note = a, c, t, g, unknown or other
  source 1..95: mol_type = other DNA
atcgtcgactgacnnnnnnnnctcgatcgctagactagctcgatcgatttcgatcgctatcgcgtagctagctannnnnnnnctgacatcgtcga

SEQ ID NO: 6 - DNA, 125 bp, synthetic construct
  modified_base 59..61: mod_base = OTHER; note = a, c, t, g, unknown or other
  modified_base 96..101: mod_base = OTHER; note = a, c, t, g, unknown or other
  source 1..125: mol_type = other DNA
aatgatacggcgaccaccgagatctacactctttccctacacgacgctcttccgatctnnnagatcggaagagcacacgtctgaactccagtcacnnnnnnatctcgtatgccgtcttctgcttg

SEQ ID NO: 7 - DNA, 42 bp, synthetic construct
  modified_base 35..42: mod_base = OTHER; note = a, c, t, g, unknown or other
  source 1..42: mol_type = other DNA
  misc_feature 1..2: note = RNA
  misc_feature 3..42: note = DNA
ttttccctacacgacgctcttccgatctagtcaannnnnnnn

SEQ ID NO: 8 - DNA, 72 bp, synthetic construct
  modified_base 1..8: mod_base = OTHER; note = a, c, t, g, unknown or other
  source 1..72: mol_type = other DNA
nnnnnnnnagatcggaagagcacacgtctgaactccagtcacgtagagatctcgtatgccgtcttctgcttg

SEQ ID NO: 9 - DNA, 27 bp, synthetic construct
  source 1..27: mol_type = other DNA
  misc_feature 1..26: note = DNA
  misc_feature 27: note = RNA
agatcggaagagcgtcgtgtagggatt

SEQ ID NO: 10 - DNA, 58 bp, synthetic construct
  source 1..58: mol_type = other DNA
aatgatacggcgaccaccgagatctacactctttccctacacgacgctcttccgatct

SEQ ID NO: 11 - DNA, 24 bp, synthetic construct
  source 1..24: mol_type = other DNA
caagcagaagacggcatacgagat

SEQ ID NO: 12 - DNA, 69 bp, synthetic construct
  modified_base 62..69: mod_base = OTHER; note = a, c, t, g, unknown or other
  source 1..69: mol_type = other DNA
  modified_base 27..29: mod_base = OTHER; note = Uracil
agatcggaagagcgtcgtgtagggattttttccctacacgacgctcttccgatctagtcaannnnnnnn

SEQ ID NO: 13 - DNA, 72 bp, synthetic construct; identical to SEQ ID NO: 8
  modified_base 1..8: mod_base = OTHER; note = a, c, t, g, unknown or other
  source 1..72: mol_type = other DNA

SEQ ID NO: 14 - DNA, 58 bp, synthetic construct; identical to SEQ ID NO: 10
  source 1..58: mol_type = other DNA